European Patent Application EP 4 814 123 A1, published September 30, 2026. Title: 一种腺病毒与CCR5-∆32突变基因重组体及其制备方法和应用. Applicant: 盛利(深圳)基因科技有限公司. Application CN. The sequence listing filed with the application follows.

SEQUENCE LISTING (4 sequences)

SEQ ID NO: 1 - DNA, 3805 bp, synthetic construct
  source 1..3805: mol_type = other DNA
tctgacatgcgatgtcgactcgactgcttcgcgatgtacgggccagatatacgcgtatctgaggggactagggtgtgtttaggcgaaaagcggggcttcggttgtacgcggttaggagtcccctcaggatatagtagtttcgcttttgcatagggagggggaaatgtagtcttatgcaatactcttgtagtcttgcaacatggtaacgatgagttagcaacatgccttacaaggagagaaaaagcaccgtgcatgagaagagctgagacatccgttcccctacaagaaactctccccgggtggaacaagatggattatcaagtgtcaagtccaatctatgacatcaattattatacatcggagccctgccaaaaaatcaatgtgaagcaaatcgcagcccgcctcctgcctccgctctactcactggtgttcatctttggttttgtgggcaacatgctggtcatcctcatcctgataaactgcaaaaggctgaagagcatgactgacatctacctgctcaacctggccatctctgacctgtttttccttcttactgtccccttctgggctcactatgctgccgcccagtgggactttggaaatacaatgtgtcaactcttgacagggctctattttataggcttcttctctggaatcttcttcatcatcctcctgacaatcgataggtacctggctgtcgtccatgctgtgtttgctttaaaagccaggacggtcacctttggggtggtgacaagtgtgatcacttgggtggtggctgtgtttgcgtctctcccaggaatcatctttaccagatctcaaaaagaaggtcttcattacacctgcagctctcattttccatacattaaagatagtcatcttggggctggtcctgccgctgcttgtcatggtcatctgctactcgggaatcctaaaaactctgcttcggtgtcgaaatgagaagaagaggcacagggctgtgaggcttatcttcaccatcatgattgtttattttctcttctgggctccctacaacattgtccttctcctgaacaccttccaggaattctttggcctgaataattgcagtagctctaacaggttggaccaagctatgcaggtgacagagactcttgggatgacgcactgctgcatcaaccccatcatctatgcctttgtcggggagaagttcagaaactacctcttagtcttcttccaaaagcacattgccaaacgcttctgcaaatgctgttctattttccagcaagaggctcccgagcgagcaagctcagtttacacccgatccactggggagcaggaaatatctgtgggcttgtgacacggactcaagtgggctggtgacccagtcagagttgtgcacatggcttagttttcatacacagcctgggctgggggtggggtgggagaggtcttttttaaaaggaagttactgttatagagggtctaagattcatccatttatttggcatctgtttaaagtagattagatcttttaagcccatcaattatagaaagccaaatcaaaatatgttgatgaaaaatagcaacctttttatctccccttcacatgcatcaagttattgacaaactctcccttcactccgaaagttccttatgtatatttaaaagaaagcctcagagaattgctgattcttgagtttagtgatctgaacagaaataccaaaattatttcagaaatgtacaactttttacctagtacaaggcaacatataggttgtaaatgtgtttaaaacaggtctttgtcttgctatggggagaaaagacatgaatatgattagtaaagaaatgacacttttcatgtgtgatttcccctccaaggtatggttaataagtttcactgacttagaaccaggcgagagacttgtggcctgggagagctggggaagcttcttaaatgagaaggaatttgagttggatcatctattgctggcaaagacagaagcctcactgcaagcactgcatgggcaagcttggctgtagaaggagacagagctggttgggaagacatggggaggaaggacaaggctagatcatgaagaaccttgacggcattgctccgtctaagtcatgagctgagcagggagatcctggttggtgttgcagaaggtttactctgtggccaaaggagggtcaggaaggatgagcatttagggcaaggagccaccaacagccctcaggtcagggtgaggatggcctctgctaagctcaaggcgtgaggatgggaaggagggaggtattcgtaaggatgggaaggagggaggtattcgtgcagcatatgaggatgcagagtcagcagaactggggtggatttgggttggaagtgagggtcagagaggagtcagagagaatccctagtcttcaagcagattggagaaacccttgaaaagacatcaagcacagaaggaggaggaggaggtttaggtcaagaagaagatggattggtgtaaaaggatgggtctggtttgcagagcttgaacacagtctcacccagactccaggctgtctttcactgaatgcttctgacttcatagatttccttcccatcccagctgaaatactgaggggtctccaggaggagactagatttatgaatacacgaggtatgaggtctaggaacatacttcagctcacacatgagatctaggtgaggattgattacctagtagtcatttcatgggttgttgggaggattctatgaggcaaccacaggcagcatttagcacatactacacattcaataagcatcaaactcttagttactcattcagggatagcactgagcaaagcattgagcaaaggggtcccatagaggtgagggaagcctgaaaaactaagatgctgcctgcccagtgcacacaagtgtaggtatcattttctgcatttaaccgtcaataggcaaaggggggaagggacatattcatttggaaataagctgccttgagccttaaaacccacaaaagtacaatttaccagcctccgtatttcagactgaatgggggtggggggggcgccttaggtacttattccagatgccttctccagacaaaccagaagcaacagaaaaaatcgtctctccctccctttgaaatgaatataccccttagtgtttgggtatattcatttcaaagggagagagagaggtttttttctgttctgtctcatatgattgtgcacatacttgagactgttttgaatttgggggatggctaaaaccatcatagtacaggtaaggtgagggaatagtaagtggtgagaactactcagggaatgaaggtgtcagaataataagaggtgctactgactttctcagcctctgaatatgaacggtgagcattgtggctgtcagcaggaagcaacgaagggaaatgtctttccttttgctcttaagttgtggagagtgcaacagtagcataggaccctaccctctgggccaagtcaaagacattctgacatcttagtatttgcatattcttatgtatgtgaaagttacaaattgcttgaaagaaaatatgcatctaataaaaaacaccttctaaaataactgtgccttctagttgccagccatctgttgtttgcccctcccccgtgccttccttgaccctggaaggtgccactcccactgtcctttcctaataaaatgaggaaattgcatcgcattgtctgagtaggtgtcattctattctggggggtggggtggggcaggacagcaagggggaggattgggaagacaatagcaggcatgctggggatgcggtgggctctatgg

SEQ ID NO: 2 - DNA, 3990 bp, synthetic construct
  source 1..3990: mol_type = other DNA
atgtttaccgccacactcgcagggtctgcacctggtgcgggtctcatcgtacctcagcaccttccagatctctgacatgcgatgtcgactcgactgcttcgcgatgtacgggccagatatacgcgtatctgaggggactagggtgtgtttaggcgaaaagcggggcttcggttgtacgcggttaggagtcccctcaggatatagtagtttcgcttttgcatagggagggggaaatgtagtcttatgcaatactcttgtagtcttgcaacatggtaacgatgagttagcaacatgccttacaaggagagaaaaagcaccgtgcatgagaagagctgagacatccgttcccctacaagaaactctccccgggtggaacaagatggattatcaagtgtcaagtccaatctatgacatcaattattatacatcggagccctgccaaaaaatcaatgtgaagcaaatcgcagcccgcctcctgcctccgctctactcactggtgttcatctttggttttgtgggcaacatgctggtcatcctcatcctgataaactgcaaaaggctgaagagcatgactgacatctacctgctcaacctggccatctctgacctgtttttccttcttactgtccccttctgggctcactatgctgccgcccagtgggactttggaaatacaatgtgtcaactcttgacagggctctattttataggcttcttctctggaatcttcttcatcatcctcctgacaatcgataggtacctggctgtcgtccatgctgtgtttgctttaaaagccaggacggtcacctttggggtggtgacaagtgtgatcacttgggtggtggctgtgtttgcgtctctcccaggaatcatctttaccagatctcaaaaagaaggtcttcattacacctgcagctctcattttccatacattaaagatagtcatcttggggctggtcctgccgctgcttgtcatggtcatctgctactcgggaatcctaaaaactctgcttcggtgtcgaaatgagaagaagaggcacagggctgtgaggcttatcttcaccatcatgattgtttattttctcttctgggctccctacaacattgtccttctcctgaacaccttccaggaattctttggcctgaataattgcagtagctctaacaggttggaccaagctatgcaggtgacagagactcttgggatgacgcactgctgcatcaaccccatcatctatgcctttgtcggggagaagttcagaaactacctcttagtcttcttccaaaagcacattgccaaacgcttctgcaaatgctgttctattttccagcaagaggctcccgagcgagcaagctcagtttacacccgatccactggggagcaggaaatatctgtgggcttgtgacacggactcaagtgggctggtgacccagtcagagttgtgcacatggcttagttttcatacacagcctgggctgggggtggggtgggagaggtcttttttaaaaggaagttactgttatagagggtctaagattcatccatttatttggcatctgtttaaagtagattagatcttttaagcccatcaattatagaaagccaaatcaaaatatgttgatgaaaaatagcaacctttttatctccccttcacatgcatcaagttattgacaaactctcccttcactccgaaagttccttatgtatatttaaaagaaagcctcagagaattgctgattcttgagtttagtgatctgaacagaaataccaaaattatttcagaaatgtacaactttttacctagtacaaggcaacatataggttgtaaatgtgtttaaaacaggtctttgtcttgctatggggagaaaagacatgaatatgattagtaaagaaatgacacttttcatgtgtgatttcccctccaaggtatggttaataagtttcactgacttagaaccaggcgagagacttgtggcctgggagagctggggaagcttcttaaatgagaaggaatttgagttggatcatctattgctggcaaagacagaagcctcactgcaagcactgcatgggcaagcttggctgtagaaggagacagagctggttgggaagacatggggaggaaggacaaggctagatcatgaagaaccttgacggcattgctccgtctaagtcatgagctgagcagggagatcctggttggtgttgcagaaggtttactctgtggccaaaggagggtcaggaaggatgagcatttagggcaaggagccaccaacagccctcaggtcagggtgaggatggcctctgctaagctcaaggcgtgaggatgggaaggagggaggtattcgtaaggatgggaaggagggaggtattcgtgcagcatatgaggatgcagagtcagcagaactggggtggatttgggttggaagtgagggtcagagaggagtcagagagaatccctagtcttcaagcagattggagaaacccttgaaaagacatcaagcacagaaggaggaggaggaggtttaggtcaagaagaagatggattggtgtaaaaggatgggtctggtttgcagagcttgaacacagtctcacccagactccaggctgtctttcactgaatgcttctgacttcatagatttccttcccatcccagctgaaatactgaggggtctccaggaggagactagatttatgaatacacgaggtatgaggtctaggaacatacttcagctcacacatgagatctaggtgaggattgattacctagtagtcatttcatgggttgttgggaggattctatgaggcaaccacaggcagcatttagcacatactacacattcaataagcatcaaactcttagttactcattcagggatagcactgagcaaagcattgagcaaaggggtcccatagaggtgagggaagcctgaaaaactaagatgctgcctgcccagtgcacacaagtgtaggtatcattttctgcatttaaccgtcaataggcaaaggggggaagggacatattcatttggaaataagctgccttgagccttaaaacccacaaaagtacaatttaccagcctccgtatttcagactgaatgggggtggggggggcgccttaggtacttattccagatgccttctccagacaaaccagaagcaacagaaaaaatcgtctctccctccctttgaaatgaatataccccttagtgtttgggtatattcatttcaaagggagagagagaggtttttttctgttctgtctcatatgattgtgcacatacttgagactgttttgaatttgggggatggctaaaaccatcatagtacaggtaaggtgagggaatagtaagtggtgagaactactcagggaatgaaggtgtcagaataataagaggtgctactgactttctcagcctctgaatatgaacggtgagcattgtggctgtcagcaggaagcaacgaagggaaatgtctttccttttgctcttaagttgtggagagtgcaacagtagcataggaccctaccctctgggccaagtcaaagacattctgacatcttagtatttgcatattcttatgtatgtgaaagttacaaattgcttgaaagaaaatatgcatctaataaaaaacaccttctaaaataactgtgccttctagttgccagccatctgttgtttgcccctcccccgtgccttccttgaccctggaaggtgccactcccactgtcctttcctaataaaatgaggaaattgcatcgcattgtctgagtaggtgtcattctattctggggggtggggtggggcaggacagcaagggggaggattgggaagacaatagcaggcatgctggggatgcggtgggctctatgggactataataataaaacgccaactttgacccggaacgcggaaaacacctgagaaaaacacctgggcgagtctccacgtaaacggtcaaagtccccgcggccctagacaaatatta

SEQ ID NO: 3 - DNA, 20 bp, synthetic construct
  source 1..20: mol_type = other DNA
agaagagctgagacatccgt

SEQ ID NO: 4 - DNA, 25 bp, synthetic construct
  source 1..25: mol_type = other DNA
ttattttagaaggtgttttttatta